European Patent Application EP 4 130 297 A1, published February 8, 2023. Title: MARKERS, PRIMERS, PROBES AND KIT FOR EARLY SCREENING AND DIAGNOSIS OF ENDOMETRIAL CANCER. Applicant: Beijing OriginPoly Bio-Tec Co.,LtD. The sequence listing filed with the application follows.

SEQUENCE LISTING (39 sequences)

SEQ ID NO: 1 - DNA, 29 bp, Artificial sequence
  based on Homo sapiens
ctaaattttttttttttttttatttagcg

SEQ ID NO: 2 - DNA, 27 bp, Artificial sequence
  based on Homo sapiens
ttaaagtgtctctcccccactttaacg

SEQ ID NO: 3 - DNA, 23 bp, Artificial sequence
  based on Homo sapiens
tataattagcgtcgcgaattata

SEQ ID NO: 4 - DNA, 25 bp, Artificial sequence
  based on Homo sapiens
aaccaagtttaaagtgattggttcg

SEQ ID NO: 5 - DNA, 25 bp, Artificial sequence
  based on Homo sapiens
aaggtccaataaaatccaccttccg

SEQ ID NO: 6 - DNA, 21 bp, Artificial sequence
  based on Homo sapiens
acccttagtcgcggggttggt

SEQ ID NO: 7 - DNA, 26 bp, Artificial sequence
  based on Homo sapiens
ataacgtttatatttttaagttatcg

SEQ ID NO: 8 - DNA, 22 bp, Artificial sequence
  based on Homo sapiens
gattagaccctctactaatccg

SEQ ID NO: 9 - DNA, 26 bp, Artificial sequence
  based on Homo sapiens
catctatttcgggcgcggagatgcgg

SEQ ID NO: 10 - DNA, 27 bp, Artificial sequence
  based on Homo sapiens
aaaaaaaatgtagttttttttttttcg

SEQ ID NO: 11 - DNA, 25 bp, Artificial sequence
  based on Homo sapiens
tttttttatttaaactaaaaaaacg

SEQ ID NO: 12 - DNA, 25 bp, Artificial sequence
  based on Homo sapiens
aatccaatgcgcgttcggattttcg

SEQ ID NO: 13 - DNA, 26 bp, Artificial sequence
  based on Homo sapiens
attccatgtatataaagatggttacg

SEQ ID NO: 14 - DNA, 24 bp, Artificial sequence
  based on Homo sapiens
gattaagaactataacttaatccg

SEQ ID NO: 15 - DNA, 25 bp, Artificial sequence
  based on Homo sapiens
atctataacgggttcggtagtagtt

SEQ ID NO: 16 - DNA, 26 bp, Artificial sequence
  based on Homo sapiens
cccaaaataagattgggttttgggcg

SEQ ID NO: 17 - DNA, 27 bp, Artificial sequence
  based on Homo sapiens
atttgaacatccccatctttcaaatcg

SEQ ID NO: 18 - DNA, 25 bp, Artificial sequence
  based on Homo sapiens
cttctagcgggcgtcgatgaagaga

SEQ ID NO: 19 - DNA, 29 bp, Artificial sequence
  based on Homo sapiens
attataaaaaataatagtatttataatcg

SEQ ID NO: 20 - DNA, 27 bp, Artificial sequence
  based on Homo sapiens
tgagttatctatttaaaataactcacg

SEQ ID NO: 21 - DNA, 24 bp, Artificial sequence
  based on Homo sapiens
tcctctgttcgttcggaggattta

SEQ ID NO: 22 - DNA, 28 bp, Artificial sequence
  based on Homo sapiens
acaataaaattaaaaagttttattgtcg

SEQ ID NO: 23 - DNA, 27 bp, Artificial sequence
  based on Homo sapiens
gttttaacaactacatctttaaaaccg

SEQ ID NO: 24 - DNA, 24 bp, Artificial sequence
  based on Homo sapiens
aaaagttcgaggcgtcgtttttgt

SEQ ID NO: 25 - DNA, 29 bp, Artificial sequence
  based on Homo sapiens
ctattaatggatttagagtattaatagcg

SEQ ID NO: 26 - DNA, 27 bp, Artificial sequence
  based on Homo sapiens
tttggttatataactaataaccaaacg

SEQ ID NO: 27 - DNA, 20 bp, Artificial sequence
  based on Homo sapiens
caatttcgtcgaattgcgcg

SEQ ID NO: 28 - DNA, 29 bp, Artificial sequence
  based on Homo sapiens
caaacacccattagggtagggtgtttgcg

SEQ ID NO: 29 - DNA, 26 bp, Artificial sequence
  based on Homo sapiens
tggtggggctaaacacccccaccacg

SEQ ID NO: 30 - DNA, 25 bp, Artificial sequence
  based on Homo sapiens
aaattcggcgcgatttcgatttgga

SEQ ID NO: 31 - DNA, 25 bp, Artificial sequence
  based on Homo sapiens
cccccactgtaagagagtgggggcg

SEQ ID NO: 32 - DNA, 28 bp, Artificial sequence
  based on Homo sapiens
ttaggttaatttaaaaaataacctaacg

SEQ ID NO: 33 - DNA, 24 bp, Artificial sequence
  based on Homo sapiens
cccccggcgcgggttcgggggatt

SEQ ID NO: 34 - DNA, 27 bp, Artificial sequence
  based on Homo sapiens
aaaactacttttggttagtagttttcg

SEQ ID NO: 35 - DNA, 26 bp, Artificial sequence
  based on Homo sapiens
tagggttaaactactataaccctacg

SEQ ID NO: 36 - DNA, 25 bp, Artificial sequence
  based on Homo sapiens
aaaaagcgttacgcgagttttttag

SEQ ID NO: 37 - DNA, 20 bp, Artificial sequence
  based on Homo sapiens
aggttaaatatagttgttga

SEQ ID NO: 38 - DNA, 17 bp, Artificial sequence
  based on Homo sapiens
caacccaaacccccaac

SEQ ID NO: 39 - DNA, 18 bp, Artificial sequence
  based on Homo sapiens
tagttgggggtttgggtt